European Patent Application EP 4 403 569 A1, published July 24, 2024. Title: ANTI-PERIOSTIN HUMANIZED MONOCLONAL ANTIBODY, AND PREPARATION METHOD THEREFOR AND USE THEREOF. Applicant: SHENYANG EYE INDUSTRY TECHNOLOGY INSTITUTE LTD. Application WO PCT/CN2022/118162, filed September 9, 2022. The sequence listing filed with the application follows.

SEQUENCE LISTING (8 sequences)

SEQ ID NO: 1 - protein, 117 aa, synthetic construct
EVQLVQSGAEVKKPGESLKISCKASGYSFTDYFMNWVRQMPGKGLEWIGRINPYSGDTLYNQRLQGQVTLSADKSISTAYLQLSSLKASDTAMYYCGRSGVSGLDYWGQGTLVTVSS

SEQ ID NO: 2 - protein, 106 aa, synthetic construct
DIQLTQSPSSLSASVGDRVTITCSASSSASYMHWYQQKPGKAPKNWIYDTSKLASGVPSRFSGSGSGTDYTLTISSLQPEDAATYYCQQWSSNPPTFGGGTKVEIK

SEQ ID NO: 3 - protein, 466 aa, synthetic construct
MKHLWFFLLLVAAPRWVLSEVQLVQSGAEVKKPGESLKISCKASGYSFTDYFMNWVRQMPGKGLEWIGRINPYSGDTLYNQRLQGQVTLSADKSISTAYLQLSSLKASDTAMYYCGRSGVSGLDYWGQGTLVTVSSASTKGPSVFPLAPSSKSTSGGTAALGCLVKDYFPEPVTVSWNSGALTSGVHTFPAVLQSSGLYSLSSVVTVPSSSLGTQTYICNVNHKPSNTKVDKKVEPKSCDKTHTCPPCPAPELLGGPSVFLFPPKPKDTLMISRTPEVTCVVVDVSHEDPEVKFNWYVDGVEVHNAKTKPREEQYNSTYRVVSVLTVLHQDWLNGKEYKCKVSNKALPAPIEKTISKAKGQPREPQVYTLPPSREEMTKNQVSLTCLVKGFYPSDIAVEWESNGQPENNYKTTPPVLDSDGSFFLYSKLTVDKSRWQQGNVFSCSVMHEALHNHYTQKSLSLSPGK

SEQ ID NO: 4 - protein, 233 aa, synthetic construct
MVLQTQVFISLLLWISGAYGDIQLTQSPSSLSASVGDRVTITCSASSSASYMHWYQQKPGKAPKNWIYDTSKLASGVPSRFSGSGSGTDYTLTISSLQPEDAATYYCQQWSSNPPTFGGGTKVEIKRTVAAPSVFIFPPSDEQLKSGTASVVCLLNNFYPREAKVQWKVDNALQSGNSQESVTEQDSKDSTYSLSSTLTLSKADYEKHKVYACEVTHQGLSSPVTKSFNRGEC

SEQ ID NO: 5 - DNA, 1401 bp, synthetic construct
  source 1..1401: mol_type = other DNA
atgaagcacctgtggttcttcctgctgctggtggctgctcctaggtgggtgctgagcgaggtgcagctggtgcagagcggcgccgaggtgaagaagcccggcgagagcctgaagatctcctgtaaggcttccggctactccttcaccgactactttatgaattgggtgcggcagatgcccggcaagggcctggagtggatcggcagaatcaatccttacagcggcgacaccctgtacaaccagcggctgcagggccaggtgaccctgtccgctgataagagcatctccaccgcctacctgcagctgtcctccctgaaggcctccgacaccgccatgtactactgtggcaggagcggcgtgagcggcctggactactggggccagggcaccctggtgaccgtgagcagcgctagcaccaagggaccttctgtgttccctctggctccttcttctaagtccacttccggtggtacagcagctctgggttgtctggtgaaggattacttcccagaaccagtgactgtgtcctggaactccggagctctgacttctggagtgcatactttcccagcagtgctgcaatctagcggactgtactctctgtcttccgtggtgactgtgccttcttcttccctggggactcaaacttacatctgcaacgtgaaccacaagccctccaacaccaaggtggacaagaaggtggagccaaagagctgcgataagacccacacctgtccaccttgtccagctccagaactgctgggtgggccttctgtgtttctgttcccacctaagccaaaggataccctgatgatctctaggaccccagaagtgacctgtgtggtcgtcgatgtgtctcatgaagaccctgaagtgaagttcaactggtacgtggacggggtggaagtgcataacgcaaagaccaagcccagggaagagcaatacaactccacctacagggtggtctccgtcctgacagtcctgcatcaggattggctgaacggcaaggagtacaagtgcaaggtctccaataaagccctgcctgcccctatcgagaaaaccattagcaaagccaaaggccagcccagggagccccaggtctatacactgccccccagcagggaggagatgacaaaaaatcaggtcagcctgacatgcctggtcaaaggcttttatcccagcgacattgccgtcgagtgggagtccaatggccagcccgagaataattataaaacaacaccccccgtcctggacagcgacggcagcttttttctgtatagcaaactgacagtcgataaaagcaggtggcagcagggcaatgtcttttcctgcagcgtcatgcacgaggccctgcacaatcactatactcagaaaagcctgagcctgtcccccgggaaatga

SEQ ID NO: 6 - DNA, 702 bp, synthetic construct
  source 1..702: mol_type = other DNA
atggtgctgcagacccaggtgtttatcagcctgctgctgtggatcagcggcgcttacggcgacatccagctgacccagtccccctccagcctgagcgctagcgtgggcgaccgggtgaccatcacctgctccgcctccagctccgccagctacatgcactggtaccagcagaagcccggcaaggcccccaagaactggatctatgataccagcaagctggccagcggcgtgcccagcagattcagcggcagcggctccggcaccgattacaccctgaccatcagctccctgcagcccgaggatgctgccacctactactgccagcagtggtcctccaacccccctacctttggcggcggcaccaaggtggagatcaagcgtacggtggctgcaccttctgtgttcatcttccctccatctgatgagcagctgaagtctggaaccgcatctgtcgtctgtctgctgaacaacttttaccccagggaggctaaggtccaatggaaggtggacaacgccctgcagtctggtaatagccaggaaagcgtgaccgaacaggattccaaggactccacctactccctgtcctccacactgacactgagcaaagccgactatgaaaagcacaaagtgtatgcctgcgaggtcactcatcagggcctgtccagccccgtgactaaaagctttaataggggggagtgctga

SEQ ID NO: 7 - DNA, 1424 bp, synthetic construct
  source 1..1424: mol_type = other DNA
gaattcgccgccaccatgaagcacctgtggttcttcctgctgctggtggctgctcctaggtgggtgctgagcgaggtgcagctggtgcagagcggcgccgaggtgaagaagcccggcgagagcctgaagatctcctgtaaggcttccggctactccttcaccgactactttatgaattgggtgcggcagatgcccggcaagggcctggagtggatcggcagaatcaatccttacagcggcgacaccctgtacaaccagcggctgcagggccaggtgaccctgtccgctgataagagcatctccaccgcctacctgcagctgtcctccctgaaggcctccgacaccgccatgtactactgtggcaggagcggcgtgagcggcctggactactggggccagggcaccctggtgaccgtgagcagcgctagcaccaagggaccttctgtgttccctctggctccttcttctaagtccacttccggtggtacagcagctctgggttgtctggtgaaggattacttcccagaaccagtgactgtgtcctggaactccggagctctgacttctggagtgcatactttcccagcagtgctgcaatctagcggactgtactctctgtcttccgtggtgactgtgccttcttcttccctggggactcaaacttacatctgcaacgtgaaccacaagccctccaacaccaaggtggacaagaaggtggagccaaagagctgcgataagacccacacctgtccaccttgtccagctccagaactgctgggtgggccttctgtgtttctgttcccacctaagccaaaggataccctgatgatctctaggaccccagaagtgacctgtgtggtcgtcgatgtgtctcatgaagaccctgaagtgaagttcaactggtacgtggacggggtggaagtgcataacgcaaagaccaagcccagggaagagcaatacaactccacctacagggtggtctccgtcctgacagtcctgcatcaggattggctgaacggcaaggagtacaagtgcaaggtctccaataaagccctgcctgcccctatcgagaaaaccattagcaaagccaaaggccagcccagggagccccaggtctatacactgccccccagcagggaggagatgacaaaaaatcaggtcagcctgacatgcctggtcaaaggcttttatcccagcgacattgccgtcgagtgggagtccaatggccagcccgagaataattataaaacaacaccccccgtcctggacagcgacggcagcttttttctgtatagcaaactgacagtcgataaaagcaggtggcagcagggcaatgtcttttcctgcagcgtcatgcacgaggccctgcacaatcactatactcagaaaagcctgagcctgtcccccgggaaatgagcggccgc

SEQ ID NO: 8 - DNA, 725 bp, synthetic construct
  source 1..725: mol_type = other DNA
gaattcgccgccaccatggtgctgcagacccaggtgtttatcagcctgctgctgtggatcagcggcgcttacggcgacatccagctgacccagtccccctccagcctgagcgctagcgtgggcgaccgggtgaccatcacctgctccgcctccagctccgccagctacatgcactggtaccagcagaagcccggcaaggcccccaagaactggatctatgataccagcaagctggccagcggcgtgcccagcagattcagcggcagcggctccggcaccgattacaccctgaccatcagctccctgcagcccgaggatgctgccacctactactgccagcagtggtcctccaacccccctacctttggcggcggcaccaaggtggagatcaagcgtacggtggctgcaccttctgtgttcatcttccctccatctgatgagcagctgaagtctggaaccgcatctgtcgtctgtctgctgaacaacttttaccccagggaggctaaggtccaatggaaggtggacaacgccctgcagtctggtaatagccaggaaagcgtgaccgaacaggattccaaggactccacctactccctgtcctccacactgacactgagcaaagccgactatgaaaagcacaaagtgtatgcctgcgaggtcactcatcagggcctgtccagccccgtgactaaaagctttaataggggggagtgctgagcggccgc